European Patent Specification EP 4 036 219 B1, published November 8, 2023. Title: BACTERIAL STRAIN AND THE USE THEREOF. Applicant: Probitat Oy. The sequence listing filed with the application follows.

SEQUENCE LISTING (5 sequences)

SEQ ID NO: 1 - DNA, 10 bp, Artificial Sequence
  primer P2
gatcggacgg

SEQ ID NO: 2 - DNA, 10 bp, Artificial Sequence
  primer P16
tcgccagcca

SEQ ID NO: 3 - DNA, 10 bp, Artificial Sequence
  Primer P17
cagacaagcc

SEQ ID NO: 4 - DNA, 20 bp, Artificial Sequence
  Primer 27f
agagtttgatcctggctcag

SEQ ID NO: 5 - DNA, 20 bp, Artificial Sequence
  Primer 685r
tctacgcatttcaccgctac